European Patent Specification EP 3 366 705 B1, published May 3, 2023. Title: FC CONTAINING POLYPEPTIDES WITH ALTERED GLYCOSYLATION AND REDUCED EFFECTOR FUNCTION. Applicant: GENZYME CORPORATION. The sequence listing filed with the application follows.

SEQUENCE LISTING (45 sequences)

SEQ ID NO: 1 - protein, 218 aa, Artificial Sequence
  Synthetic polypeptide
DIVMTQTPLSLSVTPGQPASISCKSSQSLLYSNGKTYLNWLLQKPGQSPQRLIYLVSKLDSGVPDRFSGSGSGTDFTLKISRVEAEDVGVYYCVQGTHLHTFGQGTRLEIKRTVAAPSVFIFPPSDEQLKSGTASVVCLLNNFYPREAKVQWKVDNALQSGNSQESVTEQDSKDSTYSLSSTLTLSKADYEKHKVYACEVTHQGLSSPVTKSFNRGEC

SEQ ID NO: 2 - protein, 443 aa, Artificial Sequence
  Synthetic polypeptide
VQLVESGGGLVQPGGSLRLSCAASGFTFNTYWMNWVRQAPGKGLEWVGQIRLKSNNYATHYAESVKGRFTISRDDSKNSLYLQMNSLKTEDTAVYYCTPVDFWGQGTTVTVSSASTKGPSVFPLAPSSKSTSGGTAALGCLVKDYFPEPVTVSWNSGALTSGVHTFPAVLQSSGLYSLSSVVTVPSSSLGTQTYICNVNHKPSNTKVDKKVEPKSCDKTHTCPPCPAPELLGGPSVFLFPPKPKDTLMISRTPEVTCVVVDVSHEDPEVKFNWYVDGVEVHNAKTKPREEQYNSTYRVVSVLTVLHQDWLNGKEYKCKVSNKALPAPIEKTISKAKGQPREPQVYTLPPSRDELTKNQVSLTCLVKGFYPSDIAVEWESNGQPENNYKTTPPVLDSDGSFFLYSKLTVDKSRWQQGNVFSCSVMHEALHNHYTQKSLSLSPGK

SEQ ID NO: 3 - protein, 444 aa, Artificial Sequence
  Synthetic polypeptide
EVQLVESGGGLVQPGGSLRLSCAASGFTFNTYWMNWVRQAPGKGLEWVGQIRLKSNNYATHYAESVKGRFTISRDDSKNSLYLQMNSLKTEDTAVYYCTPVDFWGQGTTVTVSSNSTKGPSVFPLAPSSKSTSGGTAALGCLVKDYFPEPVTVSWNSGALTSGVHTFPAVLQSSGLYSLSSVVTVPSSSLGTQTYICNVNHKPSNTKVDKKVEPKSCDKTHTCPPCPAPELLGGPSVFLFPPKPKDTLMISRTPEVTCVVVDVSHEDPEVKFNWYVDGVEVHNAKTKPREEQYNSTYRVVSVLTVLHQDWLNGKEYKCKVSNKALPAPIEKTISKAKGQPREPQVYTLPPSRDELTKNQVSLTCLVKGFYPSDIAVEWESNGQPENNYKTTPPVLDSDGSFFLYSKLTVDKSRWQQGNVFSCSVMHEALHNHYTQKSLSLSPGK

SEQ ID NO: 4 - protein, 444 aa, Artificial Sequence
  Synthetic polypeptide
EVQLVESGGGLVQPGGSLRLSCAASGFTFNTYWMNWVRQAPGKGLEWVGQIRLKSNNYATHYAESVKGRFTISRDDSKNSLYLQMNSLKTEDTAVYYCTPVDFWGQGTTVTVSSASTKGPSVFPLAPSSKSTSGGTAALGCLVKDYFPEPVTVSWNSGALTSGVHTFPAVLQSSGLYSLSSVVTVPSSSLGTQTYICNVNHKPSNTKVDKKVEPKSCDKTHTCPPCPAPELLGGPSVFLFPPKPKDTLMISRTPEVTCVVVDVSHEDPEVKFNWYVDGVEVHNAKTKPREEQYNSTYRVVSVLTVLHQDWLNGKEYKCKVSNKALPAPIEKTISKAKGQPREPQVYTLPPSRDELTKNQVSLTCLVKGFYPSDIAVEWESNGQPENNYKTTPPVLDSDGSFFLYSKLTVDKSRWQQGNVFSCSVMHEALHNHSTQKSLSLSPGK

SEQ ID NO: 5 - protein, 444 aa, Artificial Sequence
  Synthetic polypeptide
EVQLVESGGGLVQPGGSLRLSCAASGFTFNTYWMNWVRQAPGKGLEWVGQIRLKSNNYATHYAESVKGRFTISRDDSKNSLYLQMNSLKTEDTAVYYCTPVDFWGQGTTVTVSSASTKGPSVFPLAPSSKSTSGGTAALGCLVKDYFPEPVTVSWNSGALTSGVHTFPAVLQSSGLYSLSSVVTVPSSSLGTQTYICNVNHKPSNTKVDKKVEPKSCDKTHTCPPCPAPELLGGPSVFLFPPKPKDTLMISRTPEVTCVVVDVSHEDPEVKFNWYVDGVEVHNAKTKPREEQYNSTYRVVSVLTVLHQDWLNGKEYKCKVSNKALPAPIEKTISKAKGQPREPQVYTLPPSRDELTKNQVSLTCLVKGFYPSDIAVEWESNGQPENNYKTTPPVLDSDGSFFLYSKLTVDKSRWQQGNVFSCSVMHEALHNHYTQKNLSLSPGK

SEQ ID NO: 6 - protein, 444 aa, Artificial Sequence
  Synthetic polypeptide
EVQLVESGGGLVQPGGSLRLSCAASGFTFNTYWMNWVRQAPGKGLEWVGQIRLKSNNYATHYAESVKGRFTISRDDSKNSLYLQMNSLKTEDTAVYYCTPVDFWGQGTTVTVSSASTKGPSVFPLAPSSKSTSGGTAALGCLVKDYFPEPVTVSWNSGALTSGVHTFPAVLQSSGLYSLSSVVTVPSSSLGTQTYICNVNHKPSNTKVDKKVEPKSCDKTHTCPPCPAPELLGGPSVFLFPPKPKDTLMISRTPEVTCVVVDVSHEDPEVKFNWYVDGVEVHNAKTKPREEQYNSTYRVVSVLTVLHQDWLNGKEYKCKVSNKALPAPIEKTISKAKGQPREPQVYTLPPSRDELTKNQVSLTCLVKGFYPSDIAVEWESNGQPENNYKTTPPVLDSDGSFFLYSKLTVDKSRWQQGNVFSCSVMHEALHNHYTQKSLNLSPGK

SEQ ID NO: 7 - protein, 447 aa, Artificial Sequence
  Synthetic polypeptide
EVQLVESGGGLVQPGGSLRLSCAASGFTFNTYWMNWVRQAPGKGLEWVGQIRLKSNNYATHYAESVKGRFTISRDDSKNSLYLQMNSLKTEDTAVYYCTPVDFWGQGTTVTVSSASTKGPSVFPLAPSSKSTSGGTAALGCLVKDYFPEPVTVSWNSGALTSGVHTFPAVLQSSGLYSLSSVVTVPSSSLGTQTYICNVNHKPSNTKVDKKVEPKSCDKTHTCPPCPAPELLGGPSVFLFPPKPKDTLMISRTPEVTCVVVDVSHEDPEVKFNWYVDGVEVHNAKTKPREEQYNSTYRVVSVLTVLHQDWLNGKEYKCKVSNKALPAPIEKTISKAKGQPREPQVYTLPPSRDELTKNQVSLTCLVKGFYPSDIAVEWESNGQPENNYKTTPPVLDSDGSFFLYSKLTVDKSRWQQGNVFSCSVMHEALHNHYTQKSLSLSPGKNGT

SEQ ID NO: 8 - protein, 444 aa, Artificial Sequence
  Synthetic polypeptide
EVQLVESGGGLVQPGGSLRLSCAASGFTFNTYWMNWVRQAPGKGLEWVGQIRLKSNNYATHYAESVKGRFTISRDDSKNSLYLQMNSLKTEDTAVYYCTPVDFWGQGTTVTVSSASTKGPSVFPLAPSSKSTSGGTAALGCLVKDYFPEPVTVSWNSGALTSGVHTFPAVLQSSGLYSLSSVVTVPSSSLGTQTYICNVNHKPSNTKVDKKVEPKSCDKTHTCPPCPAPELLGGPSVFLFPPKPKDTLMISRTPEVTCVVVDVSHEDPEVKFNWYVDGVEVHNAKTKPREEQYNNTSRVVSVLTVLHQDWLNGKEYKCKVSNKALPAPIEKTISKAKGQPREPQVYTLPPSRDELTKNQVSLTCLVKGFYPSDIAVEWESNGQPENNYKTTPPVLDSDGSFFLYSKLTVDKSRWQQGNVFSCSVMHEALHNHYTQKSLSLSPGK

SEQ ID NO: 9 - protein, 215 aa, Artificial Sequence
  Synthetic polypeptide
EIVLTQSPGTLSLSPGERATLSCRASQSVSSSYLAWYQQKPGQAPRLLIYGASSRATGIPDRFSGSGSGTDFTLTISRLEPEDFAVYYCQQYGSSPWTFGQGTKVEIKRTVAAPSVFIFPPSDEQLKSGTASVVCLLNNFYPREAKVQWKVDNALQSGNSQESVTEQDSKDSTYSLSSTLTLSKADYEKHKVYACEVTHQGLSSPVTKSFNRGEC

SEQ ID NO: 10 - protein, 454 aa, Artificial Sequence
  Synthetic polypeptide
QVQLQESAPGLVKPSETLSLTCTVSGGSIRSYYWSWIRQPPGKGLEYIGYIYYTGSAIYNPSLQSRVTISVDTSKNQFSLKLNSVTAADTAVYYCAREGVRGASGYYYYGMDVWGQGTTVTVSSASTKGPSVFPLAPSSKSTSGGTAALGCLVKDYFPEPVTVSWNSGALTSGVHTFPAVLQSSGLYSLSSVVTVPSSSLGTQTYICNVNHKPSNTKVDKKVEPKSCDKTHTCPPCPAPELLGGPSVFLFPPKPKDTLMISRTPEVTCVVVDVSHEDPEVKFNWYVDGVEVHNAKTKPREEQYNSTYRVVSVLTVLHQDWLNGKEYKCKVSNKALPAPIEKTISKAKGQPREPQVYTLPPSRDELTKNQVSLTCLVKGFYPSDIAVEWESNGQPENNYKTTPPVLDSDGSFFLYSKLTVDKSRWQQGNVFSCSVMHEALHNHYTQKSLSLSPGK

SEQ ID NO: 11 - protein, 454 aa, Artificial Sequence
  Synthetic polypeptide
QVQLQESAPGLVKPSETLSLTCTVSGGSIRSYYWSWIRQPPGKGLEYIGYIYYTGSAIYNPSLQSRVTISVDTSKNQFSLKLNSVTAADTAVYYCAREGVRGASGYYYYGMDVWGQGTTVTVSSNSTKGPSVFPLAPSSKSTSGGTAALGCLVKDYFPEPVTVSWNSGALTSGVHTFPAVLQSSGLYSLSSVVTVPSSSLGTQTYICNVNHKPSNTKVDKKVEPKSCDKTHTCPPCPAPELLGGPSVFLFPPKPKDTLMISRTPEVTCVVVDVSHEDPEVKFNWYVDGVEVHNAKTKPREEQYNSTYRVVSVLTVLHQDWLNGKEYKCKVSNKALPAPIEKTISKAKGQPREPQVYTLPPSRDELTKNQVSLTCLVKGFYPSDIAVEWESNGQPENNYKTTPPVLDSDGSFFLYSKLTVDKSRWQQGNVFSCSVMHEALHNHYTQKSLSLSPGK

SEQ ID NO: 12 - protein, 214 aa, Artificial Sequence
  Synthetic polypeptide
DIQMTQSPSSLSASVGDRVTITCRASQDVNTAVAWYQQKPGKAPKLLIYSASFLYSGVPSRFSGSRSGTDFTLTISSLQPEDFATYYCQQHYTTPPTFGQGTKVEIKRTVAAPSVFIFPPSDEQLKSGTASVVCLLNNFYPREAKVQWKVDNALQSGNSQESVTEQDSKDSTYSLSSTLTLSKADYEKHKVYACEVTHQGLSSPVTKSFNRGEC

SEQ ID NO: 13 - protein, 450 aa, Artificial Sequence
  Synthetic polypeptide
EVQLVESGGGLVQPGGSLRLSCAASGFNIKDTYIHWVRQAPGKGLEWVARIYPTNGYTRYADSVKGRFTISADTSKNTAYLQMNSLRAEDTAVYYCSRWGGDGFYAMDYWGQGTLVTVSSASTKGPSVFPLAPSSKSTSGGTAALGCLVKDYFPEPVTVSWNSGALTSGVHTFPAVLQSSGLYSLSSVVTVPSSSLGTQTYICNVNHKPSNTKVDKKVEPKSCDKTHTCPPCPAPELLGGPSVFLFPPKPKDTLMISRTPEVTCVVVDVSHEDPEVKFNWYVDGVEVHNAKTKPREEQYNSTYRVVSVLTVLHQDWLNGKEYKCKVSNKALPAPIEKTISKAKGQPREPQVYTLPPSRDELTKNQVSLTCLVKGFYPSDIAVEWESNGQPENNYKTTPPVLDSDGSFFLYSKLTVDKSRWQQGNVFSCSVMHEALHNHYTQKSLSLSPGK

SEQ ID NO: 14 - protein, 450 aa, Artificial Sequence
  Synthetic polypeptide
EVQLVESGGGLVQPGGSLRLSCAASGFNIKDTYIHWVRQAPGKGLEWVARIYPTNGYTRYADSVKGRFTISADTSKNTAYLQMNSLRAEDTAVYYCSRWGGDGFYAMDYWGQGTLVTVSSNSTKGPSVFPLAPSSKSTSGGTAALGCLVKDYFPEPVTVSWNSGALTSGVHTFPAVLQSSGLYSLSSVVTVPSSSLGTQTYICNVNHKPSNTKVDKKVEPKSCDKTHTCPPCPAPELLGGPSVFLFPPKPKDTLMISRTPEVTCVVVDVSHEDPEVKFNWYVDGVEVHNAKTKPREEQYNSTYRVVSVLTVLHQDWLNGKEYKCKVSNKALPAPIEKTISKAKGQPREPQVYTLPPSRDELTKNQVSLTCLVKGFYPSDIAVEWESNGQPENNYKTTPPVLDSDGSFFLYSKLTVDKSRWQQGNVFSCSVMHEALHNHYTQKSLSLSPGK

SEQ ID NO: 15 - protein, 450 aa, Artificial Sequence
  Synthetic polypeptide
EVQLVESGGGLVQPGGSLRLSCAASGFNIKDTYIHWVRQAPGKGLEWVARIYPTNGYTRYADSVKGRFTISADTSKNTAYLQMNSLRAEDTAVYYCSRWGGDGFYAMDYWGQGTLVTVSSASTKGPSVFPLAPSSKSTSGGTAALGCLVKDYFPEPVTVSWNSGALTSGVHTFPAVLQSSGLYSLSSVVTVPSSSLGTQTYICNVNHKPSNTKVDKKVEPKSCDKTHTCPPCPAPELLGGPSVFLFPPKPKDTLMISRTPEVTCVVVDVSHEDPEVKFNWYVDGVEVHNAKTKPREEQYNNASRVVSVLTVLHQDWLNGKEYKCKVSNKALPAPIEKTISKAKGQPREPQVYTLPPSRDELTKNQVSLTCLVKGFYPSDIAVEWESNGQPENNYKTTPPVLDSDGSFFLYSKLTVDKSRWQQGNVFSCSVMHEALHNHYTQKSLSLSPGK

SEQ ID NO: 16 - protein, 450 aa, Artificial Sequence
  Synthetic polypeptide
EVQLVESGGGLVQPGGSLRLSCAASGFNIKDTYIHWVRQAPGKGLEWVARIYPTNGYTRYADSVKGRFTISADTSKNTAYLQMNSLRAEDTAVYYCSRWGGDGFYAMDYWGQGTLVTVSSNSTKGPSVFPLAPSSKSTSGGTAALGCLVKDYFPEPVTVSWNSGALTSGVHTFPAVLQSSGLYSLSSVVTVPSSSLGTQTYICNVNHKPSNTKVDKKVEPKSCDKTHTCPPCPAPELLGGPSVFLFPPKPKDTLMISRTPEVTCVVVDVSHEDPEVKFNWYVDGVEVHNAKTKPREEQYNNASRVVSVLTVLHQDWLNGKEYKCKVSNKALPAPIEKTISKAKGQPREPQVYTLPPSRDELTKNQVSLTCLVKGFYPSDIAVEWESNGQPENNYKTTPPVLDSDGSFFLYSKLTVDKSRWQQGNVFSCSVMHEALHNHYTQKSLSLSPGK

SEQ ID NO: 17-22 - skipped (6 entries)

SEQ ID NO: 23 - protein, 213 aa, Artificial Sequence
  Synthetic polypeptide
EIVLTQSPATLSLSPGERATLSCSATSSVSYMHWYQQKPGQAPRRLIYDTSKLASGVPARFSGSGSGTSYTLTISSLEPEDFAVYYCQQWSSNPLTFGGGTKVEIKRTVAAPSVFIFPPSDEQLKSGTASVVCLLNNFYPREAKVQWKVDNALQSGNSQESVTEQDSKDSTYSLSSTLTLSKADYEKHKVYACEVTHQGLSSPVTKSFNRGEC

SEQ ID NO: 24 - protein, 450 aa, Artificial Sequence
  Synthetic polypeptide
EVQLLQSGGGLVQPGGSLRLSCAASGYKFTSYVMHWVRQAPGKGLEWVGYINPYNDVTKYNEKFKGRFTLSRDNSKNTLYLQMNSLRAEDTAVYYCARGSYYDYDGFVYWGQGTLVTVSSASTKGPSVFPLAPSSKSTSGGTAALGCLVKDYFPEPVTVSWNSGALTSGVHTFPAVLQSSGLYSLSSVVTVPSSSLGTQTYICNVNHKPSNTKVDKKVEPKSCDKTHTCPPCPAPELLGGPSVFLFPPKPKDTLMISRTPEVTCVVVDVSHEDPEVKFNWYVDGVEVHNAKTKPREEQYNSTYRVVSVLTVLHQDWLNGKEYKCKVSNKALPAPIEKTISKAKGQPREPQVYTLPPSRDELTKNQVSLTCLVKGFYPSDIAVEWESNGQPENNYKTTPPVLDSDGSFFLYSKLTVDKSRWQQGNVFSCSVMHEALHNHYTQKSLSLSPGK

SEQ ID NO: 25 - protein, 450 aa, Artificial Sequence
  Synthetic polypeptide
EVQLLQSGGGLVQPGGSLRLSCAASGYKFTSYVMHWVRQAPGKGLEWVGYINPYNDVTKYNEKFKGRFTLSRDNSKNTLYLQMNSLRAEDTAVYYCARGSYYDYDGFVYWGQGTLVTVSSASTKGPSVFPLAPSSKSTSGGTAALGCLVKDYFPEPVTVSWNSGALTSGVHTFPAVLQSSGLYSLSSVVTVPSSSLGTQTYICNVNHKPSNTKVDKKVEPKSCDKTHTCPPCPAPELLGGPSVFLFPPKPKDTLMISRTPEVTCVVVDVSHEDPEVKFNWYVDGVEVHNAKTKPREEQYNNTSRVVSVLTVLHQDWLNGKEYKCKVSNKALPAPIEKTISKAKGQPREPQVYTLPPSRDELTKNQVSLTCLVKGFYPSDIAVEWESNGQPENNYKTTPPVLDSDGSFFLYSKLTVDKSRWQQGNVFSCSVMHEALHNHYTQKSLSLSPGK

SEQ ID NO: 26 - protein, 450 aa, Artificial Sequence
  Synthetic polypeptide
EVQLLQSGGGLVQPGGSLRLSCAASGYKFTSYVMHWVRQAPGKGLEWVGYINPYNDVTKYNEKFKGRFTLSRDNSKNTLYLQMNSLRAEDTAVYYCARGSYYDYDGFVYWGQGTLVTVSSASTKGPSVFPLAPSSKSTSGGTAALGCLVKDYFPEPVTVSWNSGALTSGVHTFPAVLQSSGLYSLSSVVTVPSSSLGTQTYICNVNHKPSNTKVDKKVEPKSCDKTHTCPPCPAPELLGGPSVFLFPPKPKDTLMISRTPEVTCVVVDVSHEDPEVKFNWYVDGVEVHNAKTKPREEQYNNASRVVSVLTVLHQDWLNGKEYKCKVSNKALPAPIEKTISKAKGQPREPQVYTLPPSRDELTKNQVSLTCLVKGFYPSDIAVEWESNGQPENNYKTTPPVLDSDGSFFLYSKLTVDKSRWQQGNVFSCSVMHEALHNHYTQKSLSLSPGK

SEQ ID NO: 27 - protein, 450 aa, Artificial Sequence
  Synthetic polypeptide
EVQLLQSGGGLVQPGGSLRLSCAASGYKFTSYVMHWVRQAPGKGLEWVGYINPYNDVTKYNEKFKGRFTLSRDNSKNTLYLQMNSLRAEDTAVYYCARGSYYDYDGFVYWGQGTLVTVSSASTKGPSVFPLAPSSKSTSGGTAALGCLVKDYFPEPVTVSWNSGALTSGVHTFPAVLQSSGLYSLSSVVTVPSSSLGTQTYICNVNHKPSNTKVDKKVEPKSCDKTHTCPPCPAPELLGGPSVFLFPPKPKDTLMISRTPEVTCVVVDVSHEDPEVKFNWYVDGVEVHNAKTKPREEQYQNTSRVVSVLTVLHQDWLNGKEYKCKVSNKALPAPIEKTISKAKGQPREPQVYTLPPSRDELTKNQVSLTCLVKGFYPSDIAVEWESNGQPENNYKTTPPVLDSDGSFFLYSKLTVDKSRWQQGNVFSCSVMHEALHNHYTQKSLSLSPGK

SEQ ID NO: 28 - protein, 218 aa, Artificial Sequence; identical to SEQ ID NO: 1
  Synthetic polypeptide

SEQ ID NO: 29 - protein, 444 aa, Artificial Sequence
  Synthetic polypeptide
EVQLVESGGGLVQPGGSLRLSCAASGFTFNTYWMNWVRQAPGKGLEWVGQIRLKSNNYATHYAESVKGRFTISRDDSKNSLYLQMNSLKTEDTAVYYCTPVDFWGQGTTVTVSSASTKGPSVFPLAPSSKSTSGGTAALGCLVKDYFPEPVTVSWNSGALTSGVHTFPAVLQSSGLYSLSSVVTVPSSSLGTQTYICNVNHKPSNTKVDKKVEPKSCDKTHTCPPCPAPELLGGPSVFLFPPKPKDTLMISRTPEVTCVVVDVSHEDPEVKFNWYVDGVEVHNAKTKPREEQYNSTYRVVSVLTVLHQDWLNGKEYKCKVSNKALPAPIEKTISKAKGQPREPQVYTLPPSRDELTKNQVSLTCLVKGFYPSDIAVEWESNGQPENNYKTTPPVLDSDGSFFLYSKLTVDKSRWQQGNVFSCSVMHEALHNHYTQKSLSLSPGK

SEQ ID NO: 30 - protein, 444 aa, Artificial Sequence; identical to SEQ ID NO: 8
  Synthetic polypeptide

SEQ ID NO: 31 - protein, 218 aa, Artificial Sequence
  Synthetic polypeptide
DIVMTQTPLSLSVTPGQPASISCKSSQSLLYSNGKTYLNWVLQKPGQSPQRLIYLVSKLDSGVPDRFSGSGSGTDFTLKISRVEAEDVGVYYCVQGSHFHTFGQGTKLEIKRTVAAPSVFIFPPSDEQLKSGTASVVCLLNNFYPREAKVQWKVDNALQSGNSQESVTEQDSKDSTYSLSSTLTLSKADYEKHKVYACEVTHQGLSSPVTKSFNRGEC

SEQ ID NO: 32 - protein, 444 aa, Artificial Sequence
  Synthetic polypeptide
EVQLVESGGGLVQPGGSLRLSCAASGFPFSNYWMNWVRQAPGKGLEWVGQIRLKSNNYATHYAESVKGRFTISRDDSKNSLYLQMNSLKTEDTAVYYCTPIDYWGQGTTVTVSSASTKGPSVFPLAPSSKSTSGGTAALGCLVKDYFPEPVTVSWNSGALTSGVHTFPAVLQSSGLYSLSSVVTVPSSSLGTQTYICNVNHKPSNTKVDKKVEPKSCDKTHTCPPCPAPELLGGPSVFLFPPKPKDTLMISRTPEVTCVVVDVSHEDPEVKFNWYVDGVEVHNAKTKPREEQYNSTYRVVSVLTVLHQDWLNGKEYKCKVSNKALPAPIEKTISKAKGQPREPQVYTLPPSRDELTKNQVSLTCLVKGFYPSDIAVEWESNGQPENNYKTTPPVLDSDGSFFLYSKLTVDKSRWQQGNVFSCSVMHEALHNHYTQKSLSLSPGK

SEQ ID NO: 33 - protein, 444 aa, Artificial Sequence
  Synthetic polypeptide
EVQLVESGGGLVQPGGSLRLSCAASGFPFSNYWMNWVRQAPGKGLEWVGQIRLKSNNYATHYAESVKGRFTISRDDSKNSLYLQMNSLKTEDTAVYYCTPIDYWGQGTTVTVSSASTKGPSVFPLAPSSKSTSGGTAALGCLVKDYFPEPVTVSWNSGALTSGVHTFPAVLQSSGLYSLSSVVTVPSSSLGTQTYICNVNHKPSNTKVDKKVEPKSCDKTHTCPPCPAPELLGGPSVFLFPPKPKDTLMISRTPEVTCVVVDVSHEDPEVKFNWYVDGVEVHNAKTKPREEQYNNTSRVVSVLTVLHQDWLNGKEYKCKVSNKALPAPIEKTISKAKGQPREPQVYTLPPSRDELTKNQVSLTCLVKGFYPSDIAVEWESNGQPENNYKTTPPVLDSDGSFFLYSKLTVDKSRWQQGNVFSCSVMHEALHNHYTQKSLSLSPGK

SEQ ID NO: 34 - protein, 444 aa, Artificial Sequence
  Synthetic polypeptide
EVQLVESGGGLVQPGGSLRLSCAASGFPFSNYWMNWVRQAPGKGLEWVGQIRLKSNNYATHYAESVKGRFTISRDDSKNSLYLQMNSLKTEDTAVYYCTPIDYWGQGTTVTVSSASTKGPSVFPLAPSSKSTSGGTAALGCLVKDYFPEPVTVSWNSGALTSGVHTFPAVLQSSGLYSLSSVVTVPSSSLGTQTYICNVNHKPSNTKVDKKVEPKSCDKTHTCPPCPAPELLGGPSVFLFPPKPKDTLMISRTPEVTCVVVDVSHEDPEVKFNWYVDGVEVHNAKTKPREEQYNNASRVVSVLTVLHQDWLNGKEYKCKVSNKALPAPIEKTISKAKGQPREPQVYTLPPSRDELTKNQVSLTCLVKGFYPSDIAVEWESNGQPENNYKTTPPVLDSDGSFFLYSKLTVDKSRWQQGNVFSCSVMHEALHNHYTQKSLSLSPGK

SEQ ID NO: 35 - protein, 444 aa, Artificial Sequence
  Synthetic polypeptide
EVQLVESGGGLVQPGGSLRLSCAASGFPFSNYWMNWVRQAPGKGLEWVGQIRLKSNNYATHYAESVKGRFTISRDDSKNSLYLQMNSLKTEDTAVYYCTPIDYWGQGTTVTVSSASTKGPSVFPLAPSSKSTSGGTAALGCLVKDYFPEPVTVSWNSGALTSGVHTFPAVLQSSGLYSLSSVVTVPSSSLGTQTYICNVNHKPSNTKVDKKVEPKSCDKTHTCPPCPAPELLGGPSVFLFPPKPKDTLMISRTPEVTCVVVDVSHEDPEVKFNWYVDGVEVHNAKTKPREEQYQNTSRVVSVLTVLHQDWLNGKEYKCKVSNKALPAPIEKTISKAKGQPREPQVYTLPPSRDELTKNQVSLTCLVKGFYPSDIAVEWESNGQPENNYKTTPPVLDSDGSFFLYSKLTVDKSRWQQGNVFSCSVMHEALHNHYTQKSLSLSPGK

SEQ ID NO: 36 - protein, 214 aa, Artificial Sequence; identical to SEQ ID NO: 12
  Synthetic polypeptide

SEQ ID NO: 37 - protein, 450 aa, Artificial Sequence; identical to SEQ ID NO: 13
  Synthetic polypeptide

SEQ ID NO: 38 - protein, 450 aa, Artificial Sequence; identical to SEQ ID NO: 15
  Synthetic polypeptide

SEQ ID NO: 39 - protein, 4 aa, Artificial Sequence
  Synthetic peptide
GGGG

SEQ ID NO: 40 - protein, 5 aa, Artificial Sequence
  Synthetic peptide
GGGGG

SEQ ID NO: 41 - protein, 6 aa, Artificial Sequence
  Synthetic peptide
GGGGGG

SEQ ID NO: 42 - protein, 7 aa, Artificial Sequence
  Synthetic peptide
GGGGGGG

SEQ ID NO: 43 - protein, 8 aa, Artificial Sequence
  Synthetic peptide
GGGGGGGG

SEQ ID NO: 44 - protein, 5 aa, Artificial Sequence
  Synthetic peptide
GGGGS

SEQ ID NO: 45 - protein, 10 aa, Artificial Sequence
  Synthetic peptide
GGGGSGGGGS